European Patent Application EP 4 656 659 A1, published December 3, 2025. Title: Modified scFc-engagers for treating immune diseases. Applicant: LoopLab Bio GmbH. The sequence listing filed with the application follows.

SEQUENCE LISTING (17 sequences)

SEQ ID NO: 1 - protein, 227 aa, synthetic construct
DKTHTCPPCPAXXXXXXXXXXXXPPKPKDTLMISRTPEVTCVVXXXXXXXXEVKFNWYVDGVEVHNAKTKPREEQXXXXXXVVSVLTVLHQDWLNGKEYKCKVSNXXXXXXXXXTISKAKGQPREPQVYTLPPSRDELTKNQVSLTCLVKGFYPSDIAVEWESNGQPENNYKTTPPVLDSDGSFFLYSKLTVDKSRWQQGNVFSCSVMHEALHNHYTQKSLSLSPGK

SEQ ID NO: 2 - protein, 223 aa, synthetic construct
VECPPCPAXXXXXXXXXXXPPKPKDTLMISRTPEVTCVVXXXXXXXXEVQFNWYVDGVEVHNAKTKPREEQXXXXXXVVSVLTVVHQDWLNGKEYKCKVSNXXXXXXXXXTISKTKGQPREPQVYTLPPSREEMTKNQVSLTCLVKGFYPSDISVEWESNGQPENNYKTTPPMLDSDGSFFLYSKLTVDKSRWQQGNVFSCSVMHEALHNHYTQKSLSLSPGK

SEQ ID NO: 3 - protein, 222 aa, synthetic construct
CPRCPAXXXXXXXXXXXXPPKPKDTLMISRTPEVTCVVXXXXXXXXEVQFKWYVDGVEVHNAKTKPREEQXXXXXXVVSVLTVLHQDWLNGKEYKCKVSNXXXXXXXXXTISKTKGQPREPQVYTLPPSREEMTKNQVSLTCLVKGFYPSDIAVEWESSGQPENNYNTTPPMLDSDGSFFLYSKLTVDKSRWQQGNIFSCSVMHEALHNRFTQKSLSLSPGK

SEQ ID NO: 4 - protein, 224 aa, synthetic construct
PPCPSCPAXXXXXXXXXXXXPPKPKDTLMISRTPEVTCVVXXXXXXXXEVQFNWYVDGVEVHNAKTKPREEQXXXXXXVVSVLTVLHQDWLNGKEYKCKVSNXXXXXXXXXTISKAKGQPREPQVYTLPPSQEEMTKNQVSLTCLVKGFYPSDIAVEWESNGQPENNYKTTPPVLDSDGSFFLYSRLTVDKSRWQEGNVFSCSVMHEALHNHYTQKSLSLSLGK

SEQ ID NO: 5 - protein, 232 aa, synthetic construct
EPKSCDKTHTCPPCPAXXXXXXXXXXXXPPKPKDTLMISRTPEVTCVVXXXXXXXXEVKFNWYVDGVEVHNAKTKPREEQXXXXXXVVSVLTVLHQDWLNGKEYKCKVSNXXXXXXXXXTISKAKGQPREPQVYTLPPSRDELTKNQVSLTCLVKGFYPSDIAVEWESNGQPENNYKTTPPVLDSDGSFFLYSKLTVDKSRWQQGNVFSCSVMHEALHNHYTQKSLSLSPGK

SEQ ID NO: 6 - protein, 228 aa, synthetic construct
ERKCCVECPPCPAXXXXXXXXXXXPPKPKDTLMISRTPEVTCVVXXXXXXXXEVQFNWYVDGVEVHNAKTKPREEQXXXXXXVVSVLTVVHQDWLNGKEYKCKVSNXXXXXXXXXTISKTKGQPREPQVYTLPPSREEMTKNQVSLTCLVKGFYPSDISVEWESNGQPENNYKTTPPMLDSDGSFFLYSKLTVDKSRWQQGNVFSCSVMHEALHNHYTQKSLSLSPGK

SEQ ID NO: 7 - protein, 232 aa, synthetic construct
EPKSCDTPPPCPRCPAXXXXXXXXXXXXPPKPKDTLMISRTPEVTCVVXXXXXXXXEVQFKWYVDGVEVHNAKTKPREEQXXXXXXVVSVLTVLHQDWLNGKEYKCKVSNXXXXXXXXXTISKTKGQPREPQVYTLPPSREEMTKNQVSLTCLVKGFYPSDIAVEWESSGQPENNYNTTPPMLDSDGSFFLYSKLTVDKSRWQQGNIFSCSVMHEALHNRFTQKSLSLSPGK

SEQ ID NO: 8 - protein, 229 aa, synthetic construct
ESKYGPPCPSCPAXXXXXXXXXXXXPPKPKDTLMISRTPEVTCVVXXXXXXXXEVQFNWYVDGVEVHNAKTKPREEQXXXXXXVVSVLTVLHQDWLNGKEYKCKVSNXXXXXXXXXTISKAKGQPREPQVYTLPPSQEEMTKNQVSLTCLVKGFYPSDIAVEWESNGQPENNYKTTPPVLDSDGSFFLYSRLTVDKSRWQEGNVFSCSVMHEALHNHYTQKSLSLSLGK

SEQ ID NO: 9 - protein, 665 aa, synthetic construct
MASLSRPSLPSCLCSFLLLLLLQVSSSYAGQFRVIGPRHPIRALVGDEVELPCRISPGKNATGMEVGWYRPPFSRVVHLYRNGKDQDGDQAPEYRGRTELLKDAIGEGKVTLRIRNVRFSDEGGFTCFFRDHSYQEEAAMELKVEDPFYWVSPGGGGGSGGGGSGGGGSVECPPCPAPPVAGPSVFLFPPKPKDTLMISRTPEVTCVVVDVSHEDPEVQFNWYVDGVEVHNAKTKPREEQFNSTFRVVSVLTVVHQDWLNGKEYKCKVSNKGLPAPIEKTISKTKGQPREPQVYTLPPSREEMTKNQVSLTCLVKGFYPSDISVEWESNGQPENNYKTTPPMLDSDGSFFLYSKLTVDKSRWQQGNVFSCSVMHEALHNHYTQKSLSLSPGKGGGGSGGGGSGGGGSGGGGSGGGGSGGGGSGGGGSGGGGSGGGGSGGGGSVECPPCPAPPVAGPSVFLFPPKPKDTLMISRTPEVTCVVVDVSHEDPEVQFNWYVDGVEVHNAKTKPREEQFNSTFRVVSVLTVVHQDWLNGKEYKCKVSNKGLPAPIEKTISKTKGQPREPQVYTLPPSREEMTKNQVSLTCLVKGFYPSDISVEWESNGQPENNYKTTPPMLDSDGSFFLYSKLTVDKSRWQQGNVFSCSVMHEALHNHYTQKSLSLSPGK

SEQ ID NO: 10 - protein, 897 aa, synthetic construct
MGSIGAASMEFCFDVFKELKVHHANENIFYCPIAIMSALAMVYLGAKDSTRTQINKVVRFDKLPGFGDSIEAQCGTSVNVHSSLRDILNQITKPNDVYSFSLASRLYAEERYPILPEYLQCVKELYRGGLEPINFQTAADQARELINSWVESQTNGIIRNVLQPSSVDSQTAMVLVNAIVFKGLWEKAFKDEDTQAMPFRVTEQESKPVQMMYQIGLFRVASMASEKMKILELPFASGTMSMLVLLPDEVSGLEQLESIINFEKLTEWTSSNVMEERKIKVYLPRMKMEEKYNLTSVLMAMGITDVFSSSANLSGISSAESLKISQAVHAAHAEINEAGREVVGSAEAGVDAASVSEEFRADHPFLFCIKHIATNAVLFFGRCVSPGGGGSGGGGSGGGGSVECPPCPAPPVAGPSVFLFPPKPKDTLMISRTPEVTCVVVDVSHEDPEVQFNWYVDGVEVHNAKTKPREEQFNSTFRVVSVLTVVHQDWLNGKEYKCKVSNKGLPAPIEKTISKTKGQPREPQVYTLPPSREEMTKNQVSLTCLVKGFYPSDISVEWESNGQPENNYKTTPPMLDSDGSFFLYSKLTVDKSRWQQGNVFSCSVMHEALHNHYTQKSLSLSPGKGGGGSGGGGSGGGGSGGGGSGGGGSGGGGSGGGGSGGGGSGGGGSGGGGSVECPPCPAPPVAGPSVFLFPPKPKDTLMISRTPEVTCVVVDVSHEDPEVQFNWYVDGVEVHNAKTKPREEQFNSTFRVVSVLTVVHQDWLNGKEYKCKVSNKGLPAPIEKTISKTKGQPREPQVYTLPPSREEMTKNQVSLTCLVKGFYPSDISVEWESNGQPENNYKTTPPMLDSDGSFFLYSKLTVDKSRWQQGNVFSCSVMHEALHNHYTQKSLSLSPGK

SEQ ID NO: 11 - protein, 856 aa, synthetic construct
MHSSALLCCLVLLTGVRASPGQGTQSENSCTHFPGNLPNMLRDLRDAFSRVKTFFQMKDQLDNLLLKESLLEDFKGYLGCQALSEMIQFYLEEVMPQAENQDPDIKAHVNSLGENLKTLRLRLRRCHRFLPCENKSKAVEQVKNAFNKLQEKGIYKAMSEFDIFINYIEAYMTMKIRNGGGSGGGSPGQGTQSENSCTHFPGNLPNMLRDLRDAFSRVKTFFQMKDQLDNLLLKESLLEDFKGYLGCQALSEMIQFYLEEVMPQAENQDPDIKAHVNSLGENLKTLRLRLRRCHRFLPCENKSKAVEQVKNAFNKLQEKGIYKAMSEFDIFINYIEAYMTMKIRNGGGGSGGGGSGGGGSVECPPCPAPPVAGPSVFLFPPKPKDTLMISRTPEVTCVVVDVSHEDPEVQFNWYVDGVEVHNAKTKPREEQFNSTFRVVSVLTVVHQDWLNGKEYKCKVSNKGLPAPIEKTISKTKGQPREPQVYTLPPSREEMTKNQVSLTCLVKGFYPSDISVEWESNGQPENNYKTTPPMLDSDGSFFLYSKLTVDKSRWQQGNVFSCSVMHEALHNHYTQKSLSLSPGKGGGGSGGGGSGGGGSGGGGSGGGGSGGGGSGGGGSGGGGSGGGGSGGGGSVECPPCPAPPVAGPSVFLFPPKPKDTLMISRTPEVTCVVVDVSHEDPEVQFNWYVDGVEVHNAKTKPREEQFNSTFRVVSVLTVVHQDWLNGKEYKCKVSNKGLPAPIEKTISKTKGQPREPQVYTLPPSREEMTKNQVSLTCLVKGFYPSDISVEWESNGQPENNYKTTPPMLDSDGSFFLYSKLTVDKSRWQQGNVFSCSVMHEALHNHYTQKSLSLSPGK

SEQ ID NO: 12 - protein, 48 aa, synthetic construct
CGGLERIARLEEKVKTLKAQNSELASTANMLREQVAQLKQKVMNHGGC

SEQ ID NO: 13 - protein, 53 aa, Homo sapiens
SGVRLWATRQAMLGQVHEVPEGWLIFVAEQEELYVRVQNGFRKVQLEARTPLP

SEQ ID NO: 14 - protein, 175 aa, Homo sapiens
MSSQIRQNYSTDVEAAVNSLVNLYLQASYTYLSLGFYFDRDDVALEGVSHFFRELAEEKREGYERLLKMQNQRGGRALFQDIKKPAEDEWGKTPDAMKAAMALEKKLNQALLDLHALGSARTDPHLCDFLETHFLDEEVKLIKKMGDHLTNLHRLGGPEAGLGEYLFERLTLKHD

SEQ ID NO: 15 - DNA, 1995 bp, synthetic construct
  source 1..1995: mol_type = other DNA
atggcttccctctcccgccccagcctcccttcttgcctgtgctccttcctcctgctgctgctccttcaggtgtcatcttcttatgccggacagttccgggtaattggcccaagacaccctatcagggctctggttggcgacgaagtggaattgccctgcaggatcagtcccggaaagaacgctaccggcatggaggttggttggtatagaccccctttttccagagtggttcacctctaccggaatggcaaggaccaggatggagaccaggcacctgagtatagaggtcgcactgagttgctgaaagacgcaatcggggagggtaaggtcactctccgcatcaggaacgttcggtttagcgacgagggcggttttacttgcttcttccgcgaccacagttaccaggaagaggctgctatggagctcaaggtggaggaccccttttattgggtttcccctggcggtggcggaggctctggtggcggtggcagtggcggtggaggcagtgttgagtgcccgccctgtcctgccccgcccgtcgcaggaccgagcgtttttctcttcccacccaagcccaaggatactctgatgatcagtcggacccctgaggtgacctgcgttgtggtcgatgtctcccatgaagaccctgaggttcagtttaactggtatgtggatggagttgaggtgcataatgccaaaaccaagccacgcgaggaacagtttaatagtaccttccgtgttgtatctgtcctgaccgtggtccaccaagactggctgaatggaaaagagtataaatgtaaagtgagcaacaagggcctgccagccccgatcgaaaagactatttccaagaccaagggacaaccgcgcgaaccccaagtgtacacccttccgccttcccgtgaagagatgactaagaaccaagtgtccctgacctgcctcgtgaaaggcttctatccgtccgatatctctgtagagtgggagtccaatggtcaacccgaaaataactacaaaaccactccacctatgttggattctgacggaagcttctttctttacagtaagctgacagtggacaagtcccgctggcagcaaggcaacgttttctcctgcagcgttatgcacgaggccctccacaaccactatacgcagaagtctctgtctctctcccctggcaagggcggtggcggtagcggaggcggtggctctggtggaggtggcagcggcggtggaggcagtggaggcggtggctctggaggcggaggcagcggtggcggaggcagcggcggaggtggctctggtggaggtggctctggcggaggtggcagtgtggaatgtcccccgtgccccgcgccacctgtggctggcccctccgtgttcctgtttccccctaaaccaaaagacacactcatgatttcacgcactccagaagtcacttgtgtcgtagtggacgtttctcacgaagatcccgaagtccaattcaattggtacgtcgacggcgtggaagtccacaacgcgaagacaaaaccccgtgaagagcaattcaactccacatttagggtggtcagcgtgctcacagtagtgcatcaggattggcttaacggcaaggaatacaagtgcaaggtaagtaataaaggtcttcctgctcctattgagaaaacaatctctaaaacaaaaggccagcctcgtgagcctcaggtttatactctgcctccgtctagggaggaaatgaccaaaaatcaggtctctttgacatgtctggtcaagggtttttacccttctgacatttccgtcgaatgggaaagcaacggccagccagagaacaattataagactacccccccgatgctggactccgatggttcctttttcctgtattccaaactcaccgtcgataaaagcagatggcaacagggtaatgtctttagctgtagtgtgatgcatgaagctctgcataatcattacacccaaaaatccctcagcctgtcaccagggaaa

SEQ ID NO: 16 - DNA, 2691 bp, synthetic construct
  source 1..2691: mol_type = other DNA
atgggatctatcggagcagccagcatggagttttgcttcgatgtgtttaaagagcttaaagtccaccatgccaatgaaaacattttttactgtcctattgcaattatgagcgccctggctatggtgtacctgggcgctaaggacagcacccggacgcaaatcaataaagtggtgcgctttgataagttgcccggttttggggattctatcgaagcccagtgtgggacatctgtgaatgtgcattcatctctgagagatatcctcaatcagattaccaagcctaatgacgtgtacagcttcagcctcgccagtcgattgtatgccgaagagagatacccaatcctgccagagtacctccagtgcgtaaaggaattgtatcgagggggcctggagcccatcaatttccagacagctgcagaccaggctcgggaacttatcaacagctgggtggaatcccaaaccaacggaattatcagaaacgtgcttcagccctcctctgtggactcacagactgctatggtgctggtgaacgcaattgtcttcaaggggttgtgggagaaagcttttaaagacgaagacacacaagctatgccatttcgagtcacagagcaagagagcaagcctgtacagatgatgtaccaaataggcctcttcagagtcgcaagcatggcctccgagaagatgaagattctggagctccctttcgcgagcgggacaatgagtatgctcgttcttctgcccgacgaggtgtctggactcgagcagttggaatccattattaacttcgaaaagctcacagagtggaccagttccaatgttatggaggagaggaaaatcaaggtctatctcccccggatgaagatggaagagaaatataatctcacatccgtgttgatggccatgggtatcactgacgtgttctccagtagcgccaacttgagcggcatatcctcagccgagagcctgaaaatttcccaggcagttcatgccgcccatgctgaaatcaatgaggccgggagagaggtggtagggtcagctgaagccggagtggatgcagcctccgtctccgaagaattccgggccgaccaccccttcctgttctgcattaagcatatcgctaccaacgctgtcctttttttcggccggtgtgtgtcccccggtggcggaggctctggtggcggtggcagtggcggtggaggcagtgttgagtgcccgccctgtcctgccccgcccgtcgcaggaccgagcgtttttctcttcccacccaagcccaaggatactctgatgatcagtcggacccctgaggtgacctgcgttgtggtcgatgtctcccatgaagaccctgaggttcagtttaactggtatgtggatggagttgaggtgcataatgccaaaaccaagccacgcgaggaacagtttaatagtaccttccgtgttgtatctgtcctgaccgtggtccaccaagactggctgaatggaaaagagtataaatgtaaagtgagcaacaagggcctgccagccccgatcgaaaagactatttccaagaccaagggacaaccgcgcgaaccccaagtgtacacccttccgccttcccgtgaagagatgactaagaaccaagtgtccctgacctgcctcgtgaaaggcttctatccgtccgatatctctgtagagtgggagtccaatggtcaacccgaaaataactacaaaaccactccacctatgttggattctgacggaagcttctttctttacagtaagctgacagtggacaagtcccgctggcagcaaggcaacgttttctcctgcagcgttatgcacgaggccctccacaaccactatacgcagaagtctctgtctctctcccctggcaagggcggtggcggtagcggaggcggtggctctggtggaggtggcagcggcggtggaggcagtggaggcggtggctctggaggcggaggcagcggtggcggaggcagcggcggaggtggctctggtggaggtggctctggcggaggtggcagtgtggaatgtcccccgtgccccgcgccacctgtggctggcccctccgtgttcctgtttccccctaaaccaaaagacacactcatgatttcacgcactccagaagtcacttgtgtcgtagtggacgtttctcacgaagatcccgaagtccaattcaattggtacgtcgacggcgtggaagtccacaacgcgaagacaaaaccccgtgaagagcaattcaactccacatttagggtggtcagcgtgctcacagtagtgcatcaggattggcttaacggcaaggaatacaagtgcaaggtaagtaataaaggtcttcctgctcctattgagaaaacaatctctaaaacaaaaggccagcctcgtgagcctcaggtttatactctgcctccgtctagggaggaaatgaccaaaaatcaggtctctttgacatgtctggtcaagggtttttacccttctgacatttccgtcgaatgggaaagcaacggccagccagagaacaattataagactacccccccgatgctggactccgatggttcctttttcctgtattccaaactcaccgtcgataaaagcagatggcaacagggtaatgtctttagctgtagtgtgatgcatgaagctctgcataatcattacacccaaaaatccctcagcctgtcaccagggaaa

SEQ ID NO: 17 - DNA, 2568 bp, synthetic construct
  source 1..2568: mol_type = other DNA
atgcactcatctgcgctgctttgttgcctcgttctgctgacaggcgtgcgagctagtccagggcaaggcacccaatcagaaaatagctgtacccattttcctggaaatctgccaaacatgctgcgggacctgcgggacgctttctccagagtaaagacctttttccagatgaaggaccaattggataaccttcttctgaaagaaagtctgctggaagatttcaagggataccttggctgtcaggccctcagtgagatgatccagttctatcttgaggaggttatgcctcaggcagagaatcaggacccagatataaaggcccacgtgaatagtctcggcgaaaatctcaaaacactgcggctcagacttcggcgctgccatcgcttcctgccctgcgagaataagagcaaagcagtggagcaggtgaagaacgcctttaacaaattgcaggaaaagggaatctacaaagcaatgtccgagtttgacatttttataaactacatcgaggcttatatgacaatgaaaatccgaaacggaggagggagcggagggggatctcccgggcagggtacccagtccgaaaactcatgtactcactttcccggaaacctgccaaacatgcttagggatctcagggacgctttttctcgggtcaaaacgttcttccagatgaaggatcaattggacaacctcctcctgaaagagagtttgctcgaggatttcaagggctatctgggatgtcaagctctcagcgagatgatccagttttacctggaagaagtaatgcctcaggccgagaaccaggatcctgacattaaggctcacgtgaacagcctgggcgaaaatctgaagacacttcgcctgagactcaggagatgccataggttcctgccctgtgaaaataagagtaaagctgtggagcaagtgaagaacgctttcaacaagctccaggagaaagggatttataaggcgatgagtgaattcgatattttcatcaactacatcgaggcctacatgaccatgaagatacgcaacggtggcggaggctctggtggcggtggcagtggcggtggaggcagtgttgagtgcccgccctgtcctgccccgcccgtcgcaggaccgagcgtttttctcttcccacccaagcccaaggatactctgatgatcagtcggacccctgaggtgacctgcgttgtggtcgatgtctcccatgaagaccctgaggttcagtttaactggtatgtggatggagttgaggtgcataatgccaaaaccaagccacgcgaggaacagtttaatagtaccttccgtgttgtatctgtcctgaccgtggtccaccaagactggctgaatggaaaagagtataaatgtaaagtgagcaacaagggcctgccagccccgatcgaaaagactatttccaagaccaagggacaaccgcgcgaaccccaagtgtacacccttccgccttcccgtgaagagatgactaagaaccaagtgtccctgacctgcctcgtgaaaggcttctatccgtccgatatctctgtagagtgggagtccaatggtcaacccgaaaataactacaaaaccactccacctatgttggattctgacggaagcttctttctttacagtaagctgacagtggacaagtcccgctggcagcaaggcaacgttttctcctgcagcgttatgcacgaggccctccacaaccactatacgcagaagtctctgtctctctcccctggcaagggcggtggcggtagcggaggcggtggctctggtggaggtggcagcggcggtggaggcagtggaggcggtggctctggaggcggaggcagcggtggcggaggcagcggcggaggtggctctggtggaggtggctctggcggaggtggcagtgtggaatgtcccccgtgccccgcgccacctgtggctggcccctccgtgttcctgtttccccctaaaccaaaagacacactcatgatttcacgcactccagaagtcacttgtgtcgtagtggacgtttctcacgaagatcccgaagtccaattcaattggtacgtcgacggcgtggaagtccacaacgcgaagacaaaaccccgtgaagagcaattcaactccacatttagggtggtcagcgtgctcacagtagtgcatcaggattggcttaacggcaaggaatacaagtgcaaggtaagtaataaaggtcttcctgctcctattgagaaaacaatctctaaaacaaaaggccagcctcgtgagcctcaggtttatactctgcctccgtctagggaggaaatgaccaaaaatcaggtctctttgacatgtctggtcaagggtttttacccttctgacatttccgtcgaatgggaaagcaacggccagccagagaacaattataagactacccccccgatgctggactccgatggttcctttttcctgtattccaaactcaccgtcgataaaagcagatggcaacagggtaatgtctttagctgtagtgtgatgcatgaagctctgcataatcattacacccaaaaatccctcagcctgtcaccagggaaa